European Patent Application EP 4 372 001 A1, published May 22, 2024. Title: ANTIGEN-BINDING MOLECULE SPECIFICALLY BINDING TO HGFR AND EGFR, AND PHARMACEUTICAL USE THEREOF. Applicant: JIANGSU HENGRUI PHARMACEUTICALS CO., LTD. Application WO PCT/CN2022/105714, filed July 14, 2022. The sequence listing filed with the application follows.

SEQUENCE LISTING (120 sequences)

SEQ ID NO: 1 - protein, 455 aa, synthetic construct
  REGION 1..455: note = Zal HC
QVQLVESGGGVVQPGRSLRLSCAASGFTFSTYGMHWVRQAPGKGLEWVAVIWDDGSYKYYGDSVKGRFTISRDNSKNTLYLQMNSLRAEDTAVYYCARDGITMVRGVMKDYFDYWGQGTLVTVSSASTKGPSVFPLAPSSKSTSGGTAALGCLVKDYFPEPVTVSWNSGALTSGVHTFPAVLQSSGLYSLSSVVTVPSSSLGTQTYICNVNHKPSNTKVDKRVEPKSCDKTHTCPPCPAPELLGGPSVFLFPPKPKDTLMISRTPEVTCVVVDVSHEDPEVKFNWYVDGVEVHNAKTKPREEQYNSTYRVVSVLTVLHQDWLNGKEYKCKVSNKALPAPIEKTISKAKGQPREPQVYTLPPSREEMTKNQVSLTCLVKGFYPSDIAVEWESNGQPENNYKTTPPVLDSDGSFFLYSKLTVDKSRWQQGNVFSCSVMHEALHNHYTQKSLSLSPGK

SEQ ID NO: 2 - protein, 214 aa, synthetic construct
  REGION 1..214: note = Zal LC
AIQLTQSPSSLSASVGDRVTITCRASQDISSALVWYQQKPGKAPKLLIYDASSLESGVPSRFSGSESGTDFTLTISSLQPEDFATYYCQQFNSYPLTFGGGTKVEIKRTVAAPSVFIFPPSDEQLKSGTASVVCLLNNFYPREAKVQWKVDNALQSGNSQESVTEQDSKDSTYSLSSTLTLSKADYEKHKVYACEVTHQGLSSPVTKSFNRGEC

SEQ ID NO: 3 - protein, 125 aa, synthetic construct [sequence omitted]

SEQ ID NO: 4 - protein, 107 aa, synthetic construct [sequence omitted]

SEQ ID NO: 5 - protein, 107 aa, synthetic construct
  REGION 1..107: note = Zal.1 LC variable region
DIQLTQSPSSLSASVGDRVTITCRASQDISSALVWYQQKPGKAPKLLIYDASSLESGVPSRFSGSESGTDFTLTISSLQPEDFATYYCQQFNSYPLTFGGGTKVEIK

SEQ ID NO: 6 - protein, 5 aa, synthetic construct
  REGION 1..5: note = HCDR1
TYGMH

SEQ ID NO: 7 - protein, 17 aa, synthetic construct
  REGION 1..17: note = HCDR2
VIWDDGSYKYYGDSVKG

SEQ ID NO: 8 - protein, 16 aa, synthetic construct
  REGION 1..16: note = HCDR3
DGITMVRGVMKDYFDY

SEQ ID NO: 9 - protein, 11 aa, synthetic construct
  REGION 1..11: note = LCDR1
RASQDISSALV

SEQ ID NO: 10 - protein, 7 aa, synthetic construct
  REGION 1..7: note = LCDR2
DASSLES

SEQ ID NO: 11 - protein, 9 aa, synthetic construct
  REGION 1..9: note = LCDR3
QQFNSYPLT

SEQ ID NO: 12 - protein, 119 aa, synthetic construct [sequence omitted]

SEQ ID NO: 13 - protein, 113 aa, synthetic construct [sequence omitted]

SEQ ID NO: 14 - protein, 120 aa, synthetic construct
  REGION 1..120: note = Ab10 HC variable region
QVQLVESGGGVVQPGRSLRLSCAASGFSLSNYGVHWVRQAPGKGLEWLAVIWSGGSTNYAAAFVSRLTISKDNSKNTVYLQMNSLRAEDTAVYYCARNHDNPYNYAMDYWGQGTTVTVSS

SEQ ID NO: 15 - protein, 112 aa, synthetic construct
  REGION 1..112: note = Ab10 LC variable region
DIVLTQSPDSLAVSLGERATINCRADKSVSTSTYNYLHWYQQKPGQPPKLLIYLASNLASGVPDRFSGSGSGTDFTLTISSLQAEDVAVYYCQHSRDLPPTFGQGTKLEIKR

SEQ ID NO: 16 - protein, 120 aa, synthetic construct
  REGION 1..120: note = Ab10.1 HC variable region
QVQLVESGGGVVQPGRSLRLSCAASGFSLSDYGVHWVRQAPGKGLEWLAVIWSGGSTNYADAFVSRLTISKDNSKNTVYLQMNSLRAEDTAVYYCARNHDNPYIYAMDYWGQGTTVTVSS

SEQ ID NO: 17 - protein, 111 aa, synthetic construct
  REGION 1..111: note = Ab10.1 LC variable region
DIVLTQSPDSLAVSLGERATINCRADKSVSTSTYNYLHWYQQKPGQPPKLLIYRGSFLATGVPDRFSGSGSGTDFTLTISSLQAEDVAVYYCQHSRDLPPTFGQGTKLEIK

SEQ ID NO: 18 - protein, 5 aa, synthetic construct
  REGION 1..5: note = Omab HCDR1
SYWLH

SEQ ID NO: 19 - protein, 17 aa, synthetic construct
  REGION 1..17: note = Omab HCDR2
MIDPSNSDTRFNPNFKD

SEQ ID NO: 20 - protein, 10 aa, synthetic construct
  REGION 1..10: note = Omab HCDR3
YRSYVTPLDY

SEQ ID NO: 21 - protein, 17 aa, synthetic construct
  REGION 1..17: note = Omab LCDR1
KSSQSLLYTSSQKNYLA

SEQ ID NO: 22 - protein, 7 aa, synthetic construct
  REGION 1..7: note = Omab LCDR2
WASTRES

SEQ ID NO: 23 - protein, 9 aa, synthetic construct
  REGION 1..9: note = Omab LCDR3
QQYYAYPWT

SEQ ID NO: 24 - protein, 5 aa, synthetic construct
  REGION 1..5: note = Ab10 HCDR1
NYGVH

SEQ ID NO: 25 - protein, 16 aa, synthetic construct
  REGION 1..16: note = Ab10 HCDR2
VIWSGGSTNYAAAFVS

SEQ ID NO: 26 - protein, 12 aa, synthetic construct
  REGION 1..12: note = Ab10 HCDR3
NHDNPYNYAMDY

SEQ ID NO: 27 - protein, 15 aa, synthetic construct
  REGION 1..15: note = LCDR1
RADKSVSTSTYNYLH

SEQ ID NO: 28 - protein, 7 aa, synthetic construct
  REGION 1..7: note = Ab10 LCDR2
LASNLAS

SEQ ID NO: 29 - protein, 9 aa, synthetic construct
  REGION 1..9: note = LCDR3
QHSRDLPPT

SEQ ID NO: 30 - protein, 5 aa, synthetic construct
  REGION 1..5: note = Ab10.1 HCDR1
DYGVH

SEQ ID NO: 31 - protein, 16 aa, synthetic construct
  REGION 1..16: note = Ab10.1 HCDR2
VIWSGGSTNYADAFVS

SEQ ID NO: 32 - protein, 12 aa, synthetic construct
  REGION 1..12: note = Ab10.1 HCDR3
NHDNPYIYAMDY

SEQ ID NO: 33 - protein, 7 aa, synthetic construct
  REGION 1..7: note = Ab10.1 LCDR2
RGSFLAT

SEQ ID NO: 34 - protein, 584 aa, synthetic construct
  REGION 1..584: note = EM1 chain 1
QVQLVESGGGVVQPGRSLRLSCAASGFTFSTYGMHWVRQAPGKGLEWVAVIWDDGSYKYYGDSVKGRFTISRDNSKNTLYLQMNSLRAEDTAVYYCARDGITMVRGVMKDYFDYWGQGTLVTVSSGGGGSGGGGQVQLVESGGGVVQPGRSLRLSCAASGFSLSDYGVHWVRQAPGKGLEWLAVIWSGGSTNYADAFVSRLTISKDNSKNTVYLQMNSLRAEDTAVYYCARNHDNPYIYAMDYWGQGTTVTVSSASTKGPSVFPLAPSSKSTSGGTAALGCLVKDYFPEPVTVSWNSGALTSGVHTFPAVLQSSGLYSLSSVVTVPSSSLGTQTYICNVNHKPSNTKVDKKVEPKSCDKTHTCPPCPAPELLGGPSVFLFPPKPKDTLMISRTPEVTCVVVDVSHEDPEVKFNWYVDGVEVHNAKTKPREEQYNSTYRVVSVLTVLHQDWLNGKEYKCKVSNKALPAPIEKTISKAKGQPREPQVYTLPPCREEMTKNQVSLWCLVKGFYPSDIAVEWESNGQPENNYKTTPPVLDSDGSFFLYSKLTVDKSRWQQGNVFSCSVMHEALHNHYTQKSLSLSPGK

SEQ ID NO: 35 - protein, 334 aa, synthetic construct
  REGION 1..334: note = EM1 chain 2
DIQLTQSPSSLSASVGDRVTITCRASQDISSALVWYQQKPGKAPKLLIYDASSLESGVPSRFSGSESGTDFTLTISSLQPEDFATYYCQQFNSYPLTFGGGTKVEIKGGGGSGGGGDIVLTQSPDSLAVSLGERATINCRADKSVSTSTYNYLHWYQQKPGQPPKLLIYRGSFLATGVPDRFSGSGSGTDFTLTISSLQAEDVAVYYCQHSRDLPPTFGQGTKLEIKRTVAAPSVFIFPPSDEQLKSGTASVVCLLNNFYPREAKVQWKVDNALQSGNSQESVTEQDSKDSTYSLSSTLTLSKADYEKHKVYACEVTHQGLSSPVTKSFNRGEC

SEQ ID NO: 36 - protein, 449 aa, synthetic construct
  REGION 1..449: note = EM1 chain 3
EVQLVESGGGLVQPGGSLRLSCAASGYTFTSYWLHWVRQAPGKGLEWVGMIDPSNSDTRFNPNFKDRFTISADTSKNTAYLQMNSLRAEDTAVYYCATYRSYVTPLDYWGQGTLVTVSSGGGGSGIPPKIECLPIDISIDEGKVLTVASAFTGEPTPEVTWSTGGRKIHSQEQGRFHIENTDDSTTLTIKDVQKQDGGLYTLTLRNEFGSDSATVNIHIRSIDKTHTCPPCPAPELLGGPSVFLFPPKPKDTLMISRTPEVTCVVVDVSHEDPEVKFNWYVDGVEVHNAKTKPREEQYNSTYRVVSVLTVLHQDWLNGKEYKCKVSNKALPAPIEKTISKAKGQPREPQVCTLPPSREEMTKNQVSLSCAVKGFYPSDIAVEWESNGQPENNYKTTPPVLDSDGSFFLVSKLTVDKSRWQQGNVFSCSVMHEALHNHYTQKSLSLSPGK

SEQ ID NO: 37 - protein, 215 aa, synthetic construct
  REGION 1..215: note = EM1 chain 4
DIQMTQSPSSLSASVGDRVTITCKSSQSLLYTSSQKNYLAWYQQKPGKAPKLLIYWASTRESGVPSRFSGSGSGTDFTLTISSLQPEDFATYYCQQYYAYPWTFGQGTKVEIKGGGGSSGAPRFLTRPKASVVSVGKDATLSCQIVGNPFPQVSWEKDKQPVTAGVRFRLAQDGDLYRLKILDLQLSDSGQYVCRARNAHGEAFACLGLQVDAEA

SEQ ID NO: 38 - protein, 449 aa, synthetic construct
  REGION 1..449: note = EM2 chain 1
EVQLVESGGGLVQPGGSLRLSCAASGYTFTSYWLHWVRQAPGKGLEWVGMIDPSNSDTRFNPNFKDRFTISADTSKNTAYLQMNSLRAEDTAVYYCATYRSYVTPLDYWGQGTLVTVSSASTKGPSVFPLAPSSKSTSGGTAALGCLVKDYFPEPVTVSWNSGALTSGVHTFPAVLQSSGLYSLSSVVTVPSSSLGTQTYICNVNHKPSNTKVDKKVEPKSCDKTHTCPPCPAPELLGGPSVFLFPPKPKDTLMISRTPEVTCVVVDVSHEDPEVKFNWYVDGVEVHNAKTKPREEQYNSTYRVVSVLTVLHQDWLNGKEYKCKVSNKALPAPIEKTISKAKGQPREPQVYTLPPCREEMTKNQVSLWCLVKGFYPSDIAVEWESNGQPENNYKTTPPVLDSDGSFFLYSKLTVDKSRWQQGNVFSCSVMHEALHNHYTQKSLSLSPGK

SEQ ID NO: 39 - protein, 220 aa, synthetic construct
  REGION 1..220: note = EM2 chain 2
DIQMTQSPSSLSASVGDRVTITCKSSQSLLYTSSQKNYLAWYQQKPGKAPKLLIYWASTRESGVPSRFSGSGSGTDFTLTISSLQPEDFATYYCQQYYAYPWTFGQGTKVEIKRTVAAPSVFIFPPSDEQLKSGTASVVCLLNNFYPREAKVQWKVDNALQSGNSQESVTEQDSKDSTYSLSSTLTLSKADYEKHKVYACEVTHQGLSSPVTKSFNRGEC

SEQ ID NO: 40 - protein, 455 aa, synthetic construct
  REGION 1..455: note = EM2 chain 3
QVQLVESGGGVVQPGRSLRLSCAASGFTFSTYGMHWVRQAPGKGLEWVAVIWDDGSYKYYGDSVKGRFTISRDNSKNTLYLQMNSLRAEDTAVYYCARDGITMVRGVMKDYFDYWGQGTLVTVSSGGGGSGIPPKIECLPIDISIDEGKVLTVASAFTGEPTPEVTWSTGGRKIHSQEQGRFHIENTDDSTTLTIKDVQKQDGGLYTLTLRNEFGSDSATVNIHIRSIDKTHTCPPCPAPELLGGPSVFLFPPKPKDTLMISRTPEVTCVVVDVSHEDPEVKFNWYVDGVEVHNAKTKPREEQYNSTYRVVSVLTVLHQDWLNGKEYKCKVSNKALPAPIEKTISKAKGQPREPQVCTLPPSREEMTKNQVSLSCAVKGFYPSDIAVEWESNGQPENNYKTTPPVLDSDGSFFLVSKLTVDKSRWQQGNVFSCSVMHEALHNHYTQKSLSLSPGK

SEQ ID NO: 41 - protein, 209 aa, synthetic construct
  REGION 1..209: note = EM2 chain 4
DIQLTQSPSSLSASVGDRVTITCRASQDISSALVWYQQKPGKAPKLLIYDASSLESGVPSRFSGSESGTDFTLTISSLQPEDFATYYCQQFNSYPLTFGGGTKVEIKGGGGSSGAPRFLTRPKASVVSVGKDATLSCQIVGNPFPQVSWEKDKQPVTAGVRFRLAQDGDLYRLKILDLQLSDSGQYVCRARNAHGEAFACLGLQVDAEA

SEQ ID NO: 42 - protein, 627 aa, synthetic construct
  REGION 1..627: note = EGFR-His
LEEKKVCQGTSNKLTQLGTFEDHFLSLQRMFNNCEVVLGNLEITYVQRNYDLSFLKTIQEVAGYVLIALNTVERIPLENLQIIRGNMYYENSYALAVLSNYDANKTGLKELPMRNLQEILHGAVRFSNNPALCNVESIQWRDIVSSDFLSNMSMDFQNHLGSCQKCDPSCPNGSCWGAGEENCQKLTKIICAQQCSGRCRGKSPSDCCHNQCAAGCTGPRESDCLVCRKFRDEATCKDTCPPLMLYNPTTYQMDVNPEGKYSFGATCVKKCPRNYVVTDHGSCVRACGADSYEMEEDGVRKCKKCEGPCRKVCNGIGIGEFKDSLSINATNIKHFKNCTSISGDLHILPVAFRGDSFTHTPPLDPQELDILKTVKEITGFLLIQAWPENRTDLHAFENLEIIRGRTKQHGQFSLAVVSLNITSLGLRSLKEISDGDVIISGNKNLCYANTINWKKLFGTSGQKTKIISNRGENSCKATGQVCHALCSPEGCWGPEPRDCVSCRNVSRGRECVDKCNLLEGEPREFVENSECIQCHPECLPQAMNITCTGRGPDNCIQCAHYIDGPHCVKTCPAGVMGENNTLVWKYADAGHVCHLCHPNCTYGCTGPGLEGCPTNGPKIPSHHHHHH

SEQ ID NO: 43 - protein, 914 aa, synthetic construct
  REGION 1..914: note = HGFR-His
ECKEALAKSEMNVNMKYQLPNFTAETPIQNVILHEHHIFLGATNYIYVLNEEDLQKVAEYKTGPVLEHPDCFPCQDCSSKANLSGGVWKDNINMALVVDTYYDDQLISCGSVNRGTCQRHVFPHNHTADIQSEVHCIFSPQIEEPSQCPDCVVSALGAKVLSSVKDRFINFFVGNTINSSYFPDHPLHSISVRRLKETKDGFMFLTDQSYIDVLPEFRDSYPIKYVHAFESNNFIYFLTVQRETLDAQTFHTRIIRFCSINSGLHSYMEMPLECILTEKRKKRSTKKEVFNILQAAYVSKPGAQLARQIGASLNDDILFGVFAQSKPDSAEPMDRSAMCAFPIKYVNDFFNKIVNKNNVRCLQHFYGPNHEHCFNRTLLRNSSGCEARRDEYRTEFTTALQRVDLFMGQFSEVLLTSISTFIKGDLTIANLGTSEGRFMQVVVSRSGPSTPHVNFLLDSHPVSPEVIVEHTLNQNGYTLVITGKKITKIPLNGLGCRHFQSCSQCLSAPPFVQCGWCHDKCVRSEECLSGTWTQQICLPAIYKVFPNSAPLEGGTRLTICGWDFGFRRNNKFDLKKTRVLLGNESCTLTLSESTMNTLKCTVGPAMNKHFNMSIIISNGHGTTQYSTFSYVDPVITSISPKYGPMAGGTLLTLTGNYLNSGNSRHISIGGKTCTLKSVSNSILECYTPAQTISTEFAVKLKIDLANRETSIFSYREDPIVYEIHPTKSFISGGSTITGVGKNLNSVSVPRMVINVHEAGRNFTVACQHRSNSEIICCTTPSLQQLNLQLPLKTKAFFMLDGILSKYFDLIYVHNPVFKPFEKPVMISMGNENVLEIKGNDIDPEAVKGEVLKVGNKSCENIHLHSEAVLCTVPNDLLKLNSELNIEWKQAISSTVLGKVIVQPDQNFTHHHHHH

SEQ ID NO: 44 - protein, 703 aa, synthetic construct
  REGION 1..703: note = HGF-His
QRKRRNTIHEFKKSAKTTLIKIDPALKIKTKKVNTADQCANRCTRNKGLPFTCKAFVFDKARKQCLWFPFNSMSSGVKKEFGHEFDLYENKDYIRNCIIGKGRSYKGTVSITKSGIKCQPWSSMIPHEHSFLPSSYRGKDLQENYCRNPRGEEGGPWCFTSNPEVRYEVCDIPQCSEVECMTCNGESYRGLMDHTESGKICQRWDHQTPHRHKFLPERYPDKGFDDNYCRNPDGQPRPWCYTLDPHTRWEYCAIKTCADNTMNDTDVPLETTECIQGQGEGYRGTVNTIWNGIPCQRWDSQYPHEHDMTPENFKCKDLRENYCRNPDGSESPWCFTTDPNIRVGYCSQIPNCDMSHGQDCYRGNGKNYMGNLSQTRSGLTCSMWDKNMEDLHRHIFWEPDASKLNENYCRNPDDDAHGPWCYTGNPLIPWDYCPISRCEGDTTPTIVNLDHPVISCAKTKQLRVVNGIPTRTNIGWMVSLRYRNKHICGGSLIKESWVLTARQCFPSRDLKDYEAWLGIHDVHGRGDEKCKQVLNVSQLVYGPEGSDLVLMKLARPAVLDDFVSTIDLPNYGCTIPEKTSCSVYGWGYTGLINYDGLLRVAHLYIMGNEKCSQHHRGKVTLNESEICAGAEKIGSGPCEGDYGGPLVCEQHKMRMVLGVIVPGRGCAIPNRPGIFVRVAYYAKWIHKIILTYKVPQSHHHHHH

SEQ ID NO: 45 - protein, 98 aa, synthetic construct
  REGION 1..98: note = T.0
GIPPKIEALPSDISIDEGKVLTVACAFTGEPTPEVTWSCGGRKIHSQEQGRFHIENTDDLTTLIIMDVQKQDGGLYTLSLGNEFGSDSATVNIHIRSI

SEQ ID NO: 46 - protein, 98 aa, synthetic construct
  REGION 1..98: note = T.1
GIPPKIECLPSDISIDEGKVLTVASAFTGEPTPEVTWSTGGRKIHSQEQGRFHIENTDDLTTLIIMDVQKQDGGLYTLSLGNEFGSDSATVNIHIRSI

SEQ ID NO: 47 - protein, 98 aa, synthetic construct
  REGION 1..98: note = T.2
GIPPKIEALPSDISIDEGKCLTVASAFTGEPTPEVTWSTGGRKIHSQEQGRFHIENTDDLTTLIIMDVQKQDGGLYTLSLGNEFGSDSATVNIHIRSI

SEQ ID NO: 48 - protein, 98 aa, synthetic construct
  REGION 1..98: note = T.3
GIPPKIEALPSDISIDEGKVLTVASCFTGEPTPEVTWSTGGRKIHSQEQGRFHIENTDDLTTLIIMDVQKQDGGLYTLSLGNEFGSDSATVNIHIRSI

SEQ ID NO: 49 - protein, 98 aa, synthetic construct
  REGION 1..98: note = T.4
GIPPKIEALPSDISIDEGKVLCVASAFTGEPTPEVTWSTGGRKIHSQEQGRFHIENTDDLTTLIIMDVQKQDGGLYTLSLGNEFGSDSATVNIHIRSI

SEQ ID NO: 50 - protein, 103 aa, synthetic construct
  REGION 1..103: note = T.5
KAGIRGIPPKIECLPSDISIDEGKVLTVASAFTGEPTPEVTWSTGGRKIHSQEQGRFHIENTDDLTTLIIMDVQKQDGGLYTLSLGNEFGSDSATVNIHIRSI

SEQ ID NO: 51 - protein, 103 aa, synthetic construct
  REGION 1..103: note = T.6
KAGIRGIPPKIEALPSDISIDEGKVLTVACAFTGEPTPEVTWSCGGRKIHSQEQGRFHIENTDDLTTLIIMDVQKQDGGLYTLSLGNEFGSDSATVNIHIRSI

SEQ ID NO: 52 - protein, 98 aa, synthetic construct
  REGION 1..98: note = T.7
GIPPKIECLPSDISIDEGKVLTVASAFTGEPTPEVTWSTGGRKIHSQEQGRFHIENTDDLTTLIISDVQKQDGGLYSLSLGNEFGSDSATVNIHIRSI

SEQ ID NO: 53 - protein, 98 aa, synthetic construct
  REGION 1..98: note = T.8
GIPPKIECLPSDISIDEGKVLTVASAFTGEPTPEVTWSTGGRKIHSQEQGRFHIENTDDLTTLIIKDVQRQDGGLYTLTLRNEFGSDSATVNIHIRSI

SEQ ID NO: 54 - protein, 98 aa, synthetic construct
  REGION 1..98: note = T.9
GIWPKIECLPIDLSIDEGKVLMVASAFTGEPTPEVTWSTGGRKIHSQEQGRFHIENTDDLTTLIIMDVQKQDGGLYTLSLGMEFGSDSATVNIHIRSI

SEQ ID NO: 55 - protein, 98 aa, synthetic construct
  REGION 1..98: note = T.10
GIPPKIECLPIDISIDEGKVLTVASAFTGEPTPEVTWSTGGRKIHSQEQGRFHIENTDDLTTLIIKDVQKQDGGLYTLTLRNEFGSDSATVNIHIRSI

SEQ ID NO: 56 - protein, 98 aa, synthetic construct
  REGION 1..98: note = T.11
GIPPKIECLPSDISIDEGKVLTVASAFTGEPTPEVTWSTSGKKISSEEGGRFHIESTEDLTTLIIMDVQKQDGGVYTLSLGNDLGSDSATVNIHIRSI

SEQ ID NO: 57 - protein, 98 aa, synthetic construct
  REGION 1..98: note = T.12
GIPPKIECLPSDISIDEGKVLTVASAFTGEPTPEVTWSTGGRKIHSEEGGRFHIESTEDLTTLIIMDVQKQDGGVYTLSLGNEFGSDSATVNIHIRSI

SEQ ID NO: 58 - protein, 98 aa, synthetic construct
  REGION 1..98: note = T.13
GIPPKIECLPSDISIDEGKVLTVASAFTGEPTPEVTWSTGGRKIHSQEQGRFHIESTEDLTTLIIMDVQKQDGGVYTLSLGNEFGSDSATVNIHIRSI

SEQ ID NO: 59 - protein, 98 aa, synthetic construct
  REGION 1..98: note = T.14
GIPPKIECLPSDISIDEGKVLTVASAFTGEPTPEVTWSTGGRKIHSQEQGRFHIESTEDLTTLIISDVQKQDGGLYSLSLGNEFGSDSATVNIHIRSI

SEQ ID NO: 60 - protein, 103 aa, synthetic construct
  REGION 1..103: note = T.15
KAGIRGIPPKIECLPSDISIDEGKVLTVASAFTGEPTPEVTWSTGGRKIHSQEQGRFHIESTEDLTTLIISDVQKQDGGLYSLSLGNEFGSDSATVNIHIRSI

SEQ ID NO: 61 - protein, 98 aa, synthetic construct
  REGION 1..98: note = T.16
GIPPKIECLPIDISIDEGKVLTVASAFTGEPTPEVTWSTGGRKIHSQEQGRFHIENTDDSTTLTIKDVQKQDGGLYTLTLRNEFGSDSATVNIHIRSI

SEQ ID NO: 62 - protein, 98 aa, synthetic construct
  REGION 1..98: note = T.17
GIPPKIECLPIDISIDEGKCLTVASAFTGEPTPEVTWSTGGRKIHSQEQGRFHIENTDDSTTLTIKDVQKQDGGLYTLTLRNEFGSDSATVNIHIRSI

SEQ ID NO: 63 - protein, 98 aa, synthetic construct
  REGION 1..98: note = T.18
GIPPKIECLPIDISIDEGKVLTVASCFTGEPTPEVTWSTGGRKIHSQEQGRFHIENTDDSTTLTIKDVQKQDGGLYTLTLRNEFGSDSATVNIHIRSI

SEQ ID NO: 64 - protein, 97 aa, synthetic construct
  REGION 1..97: note = O.0
SGAPRFLTRPKAFVVSVGKDATLSCQIVGNPTPQVSWEKDQQPVAAGARFRLAQDGDLYRLTILDLALGDSGQYVCRARNAIGEAFAAVGLQVDAEA

SEQ ID NO: 65 - protein, 98 aa, synthetic construct
  REGION 1..98: note = OL.0
QGSPPCFLRFPRPVRVVSGAEAELKCVVLGEPPPVVVWEKGGQQLAASERLSFPADGAEHGLLLTAALPTDAGVYVCRARNAAGEAYAAAAVTVLEPP

SEQ ID NO: 66 - protein, 97 aa, synthetic construct
  REGION 1..97: note = O.1
SGAPRFLTRPKAFVVSVGKDATLSCQIVGNPTPQVSWEKDQQPVAAGARFRLAQDGDLYRLTILDLALGDSGQYVCRARNAIGEAFACVGLQVDAEA

SEQ ID NO: 67 - protein, 97 aa, synthetic construct
  REGION 1..97: note = O.2
SGCPRFLTRPKAFVVSVGKDATLSCQIVGNPTPQVSWEKDQQPVAAGARFRLAQDGDLYRLTILDLALGDSGQYVCRARNAIGEAFAAVGLQVDAEA

SEQ ID NO: 68 - protein, 97 aa, synthetic construct
  REGION 1..97: note = O.3
SGAPRFLTCPKAFVVSVGKDATLSCQIVGNPTPQVSWEKDQQPVAAGARFRLAQDGDLYRLTILDLALGDSGQYVCRARNAIGEAFAAVGLQVDAEA

SEQ ID NO: 69 - protein, 97 aa, synthetic construct
  REGION 1..97: note = O.4
SGAPRFLTRPKAFVVSVGKDATLSSQIVGNPTPQVSWEKDQQPVAAGARFRLAQDGDLYRLTILDLALGDSGQYVSRARNAIGEAFACVGLQVDAEA

SEQ ID NO: 70 - protein, 97 aa, synthetic construct
  REGION 1..97: note = O.5
SGCPRFLTRPKAFVVSVGKDATLSSQIVGNPTPQVSWEKDQQPVAAGARFRLAQDGDLYRLTILDLALGDSGQYVSRARNAIGEAFAAVGLQVDAEA

SEQ ID NO: 71 - protein, 97 aa, synthetic construct
  REGION 1..97: note = O.6
SGAPRFLTCPKAFVVSVGKDATLSSQIVGNPTPQVSWEKDQQPVAAGARFRLAQDGDLYRLTILDLALGDSGQYVSRARNAIGEAFAAVGLQVDAEA

SEQ ID NO: 72 - protein, 97 aa, synthetic construct
  REGION 1..97: note = O.7
SGAPRFKTRPKAFVVSVGKDATLSSQIVGNPTPQVSWEKDQQPVAAGARFRLAQDGDLYRLKILDLALGDSGQYVSRARNAIGEAFACVGLQVDAEA

SEQ ID NO: 73 - protein, 97 aa, synthetic construct
  REGION 1..97: note = O.8
SGAPRFKTRPKAFVVSVGKDATLSSQIVGNPTPQVSWEKDQQPVAAGARFRLAQDGDLYRLHILDLALGDSGQYVSRARNAIGEAFACVGLQVDAEA

SEQ ID NO: 74 - protein, 97 aa, synthetic construct
  REGION 1..97: note = O.9
SGAPRFLTRPLAFVVSVGKDATLSSQIVGNPTPQVSWEKDQQPVAAGARFRLAQDGDLYRLKILDLALGDSGQYVSRARNAIGEAFACVGLQVDAEA

SEQ ID NO: 75 - protein, 97 aa, synthetic construct
  REGION 1..97: note = O.10
SGAPRFLTRPLAFVVSVGKDATLSSQIVGNPTPQVSWEKDQQPVAAGARFRLAQDGDLYRLHILDLALGDSGQYVSRARNAIGEAFACVGLQVDAEA

SEQ ID NO: 76 - protein, 102 aa, synthetic construct
  REGION 1..102: note = O.11
DQPQFSGAPRFLTRPKAFVVSVGKDATLSSQIVGNPTPQVSWEKDQQPVAAGARFRLAQDGDLYRLTILDLALGDSGQYVSRARNAIGEAFACVGLQVDAEA

SEQ ID NO: 77 - protein, 102 aa, synthetic construct
  REGION 1..102: note = O.12
DQPQFSGAPRFKTRPKAFVVSVGKDATLSSQIVGNPTPQVSWEKDQQPVAAGARFRLAQDGDLYRLKILDLALGDSGQYVSRARNAIGEAFACVGLQVDAEA

SEQ ID NO: 78 - protein, 102 aa, synthetic construct
  REGION 1..102: note = O.13
DQPQFSGAPRFKTRPKAFVVSVGKDATLSSQIVGNPTPQVSWEKDQQPVAAGARFRLAQDGDLYRLHILDLALGDSGQYVSRARNAIGEAFACVGLQVDAEA

SEQ ID NO: 79 - protein, 102 aa, synthetic construct
  REGION 1..102: note = O.14
DQPQFSGAPRFRTRPKAFVVSVGKDATLSSQIVGNPTPQVSWEKDQQPVAAGARFRLAQDGDLYRLKILDLALGDSGQYVSRARNAIGEAFACVGLQVDAEA

SEQ ID NO: 80 - protein, 102 aa, synthetic construct
  REGION 1..102: note = O.15
DQPQFSGAPRFRTRPKAFVVSVGKDATLSSQIVGNPTPQVSWEKDQQPVAAGARFRLAQDGDLYRLHILDLALGDSGQYVSRARNAIGEAFACVGLQVDAEA

SEQ ID NO: 81 - protein, 102 aa, synthetic construct
  REGION 1..102: note = O.16
DQPQFSGAPRFLTRPKAFVVSVGKDATLSCQIVGNPTPQVSWEKDQQPVAAGARFRLAQDGDLYRLTILDLALGDSGQYVCRARNAIGEAFAAVGLQVDAEA

SEQ ID NO: 82 - protein, 98 aa, synthetic construct
  REGION 1..98: note = OL.1
QGSPPEFLRFPRPVRVVSGAEAELKCVVLGEPPPVVVWEKGGQQLAASERLSFPADGAEHGLLLTAALPTDAGCYVCRARNAAGEAYAAAAVTVLEPP

SEQ ID NO: 83 - protein, 98 aa, synthetic construct
  REGION 1..98: note = OL.2
QGSPPEFLRFPRPVRVVSGAEAELKCVVLGEPPPVVVWEKGGQQLAASERLSFPADGAEHGLLLTAALPTDAGVYVCRARNAACEAYAAAAVTVLEPP

SEQ ID NO: 84 - protein, 98 aa, synthetic construct
  REGION 1..98: note = OL.3
QGSPPEFLRFPRPVRVVSGAEAELKCVVLGEPPPVVVWEKGGQQLAASERLSFPADGAEHGLLLTAALPTDAGVYVCRARNAAGECYAAAAVTVLEPP

SEQ ID NO: 85 - protein, 98 aa, synthetic construct
  REGION 1..98: note = OL.4
QGSPPEFLRFPRPVRVVSGAEAELKSVVLGEPPPVVVWEKGGQQLAASERLSFPADGAEHGLLLTAALPTDAGCYVSRARNAAGEAYAAAAVTVLEPP

SEQ ID NO: 86 - protein, 98 aa, synthetic construct
  REGION 1..98: note = OL.5
QGSPPEFLRFPRPVRVVSGAEAELKSVVLGEPPPVVVWEKGGQQLAASERLSFPADGAEHGLLLTAALPTDAGVYVSRARNAACEAYAAAAVTVLEPP

SEQ ID NO: 87 - protein, 98 aa, synthetic construct
  REGION 1..98: note = OL.6
QGSPPEFLRFPRPVRVVSGAEAELKSVVLGEPPPVVVWEKGGQQLAASERLSFPADGAEHGLLLTAALPTDAGVYVSRARNAAGECYAAAAVTVLEPP

SEQ ID NO: 88 - protein, 97 aa, synthetic construct
  REGION 1..97: note = O.17
SGAPRFLTRPKSYTVSVGKDASLSSQIVGNPTPQVSWEKDQQPVAAGARFRLAQDGDLYRLKILDLALGDSGQYVSRARNAIGEAFACVGLQVDAEA

SEQ ID NO: 89 - protein, 97 aa, synthetic construct
  REGION 1..97: note = O.18
SEAPRFLTRPLAFVVSEGKDATLSSQIVGDPPPEVTWEKDQQPITAGARFRLAQDGDVYRLEILDLQLSDSGQYVSRARNAIGEAFACVGLQVDAEG

SEQ ID NO: 90 - protein, 97 aa, synthetic construct
  REGION 1..97: note = O.19
SGAPRFLTRPLAFVVSVGKLAMLSSQIVGNPTPQVSWEKDQQPVAAGARFRLLQDGDLYRLKILDLALGDSGQYVSRARNAIGEAFACVGLQVDAEA

SEQ ID NO: 91 - protein, 97 aa, synthetic construct
  REGION 1..97: note = O.20
SGAPRFLTRPLAFVVSVGKDATLSSQIVGNPTPQVSWEKDKQPVTAGARFRLAQDGDLYRLKILDLQLSDSGQYVSRARNAIGEAFACLGLQVDAEA

SEQ ID NO: 92 - protein, 97 aa, synthetic construct
  REGION 1..97: note = O.21
SGAPRFLTRPLAFVVSVGKDATLSSQIVGNPTPQVSWEKDQLPVTAGARFRLAQDGDLYRLKILDLTLSDSGQYVSRARNAIGEAFACVGLEVGAEA

SEQ ID NO: 93 - protein, 97 aa, synthetic construct
  REGION 1..97: note = O.22
SGAPRFLTRPLSYVVSVGKDASLSSQIVGNPTPQVSWEKDQLPVTAGARFRLAQDGDLYRLKILDLQLSDSGQYVSRARNAIGEAFACVGLEVGAEA

SEQ ID NO: 94 - protein, 102 aa, synthetic construct
  REGION 1..102: note = O.23
DQPQFSGAPRFLTRPLSYVVSVGKDASLSSQIVGNPTPQVSWEKDQLPVTAGARFRLAQDGDLYRLKILDLQLSDSGQYVSRARNAIGEAFACVGLEVGAEA

SEQ ID NO: 95 - protein, 97 aa, synthetic construct
  REGION 1..97: note = O.24
SGAPRFLTRPKAFVVSVGKDATLSSQIVGNPFPQVSWEKDKQPVTAGVRFRLAQDGDLYRLKILDLQLSDSGQYVSRARNAIGEAFACLGLQVDAEA

SEQ ID NO: 96 - protein, 97 aa, synthetic construct
  REGION 1..97: note = O.25
SGAPRFLTRPKASVVSVGKDATLSSQIVGNPFPQVSWEKDKQPVTAGVRFRLAQDGDLYRLKILDLQLSDSGQYVSRARNAHGEAFACLGLQVDAEA

SEQ ID NO: 97 - protein, 97 aa, synthetic construct
  REGION 1..97: note = O.26
SGCPRFLTRPKASVVSVGKDATLSSQIVGNPFPQVSWEKDKQPVTAGVRFRLAQDGDLYRLKILDLQLSDSGQYVSRARNAHGEAFACLGLQVDAEA

SEQ ID NO: 98 - protein, 97 aa, synthetic construct
  REGION 1..97: note = O.27
SGAPRFLTCPKASVVSVGKDATLSSQIVGNPFPQVSWEKDKQPVTAGVRFRLAQDGDLYRLKILDLQLSDSGQYVSRARNAHGEAFACLGLQVDAEA

SEQ ID NO: 99 - protein, 97 aa, synthetic construct
  REGION 1..97: note = O.28
SGAPRFLTRPKASVVSVGKDATLSCQIVGNPFPQVSWEKDKQPVTAGVRFRLAQDGDLYRLKILDLQLSDSGQYVCRARNAHGEAFACLGLQVDAEA

SEQ ID NO: 100 - protein, 97 aa, synthetic construct
  REGION 1..97: note = O.29
SGCPRFLTRPKASVVSVGKDATLSCQIVGNPFPQVSWEKDKQPVTAGVRFRLAQDGDLYRLKILDLQLSDSGQYVCRARNAHGEAFACLGLQVDAEA

SEQ ID NO: 101 - protein, 97 aa, synthetic construct
  REGION 1..97: note = O.30
SGAPRFLTCPKASVVSVGKDATLSCQIVGNPFPQVSWEKDKQPVTAGVRFRLAQDGDLYRLKILDLQLSDSGQYVCRARNAHGEAFACLGLQVDAEA

SEQ ID NO: 102 - protein, 97 aa, synthetic construct
  REGION 1..97: note = O.31
SGAPRFLTRPKASVVSVGKDATLSSQIVGNPFPQVSWEKDKQPVTAGVRFRLAQDGDLYRLKILDCQLSDSGQYVSRARNAHGEAFACLGLQCDAEA

SEQ ID NO: 103 - protein, 97 aa, synthetic construct
  REGION 1..97: note = O.32
SGCPRFLTRPKASVVSVGKDATLSSQIVGNPFPQVSWEKDKQPVTAGVRFRLAQDGDLYRLKILDCQLSDSGQYVSRARNAHGEAFACLGLQCDAEA

SEQ ID NO: 104 - protein, 97 aa, synthetic construct
  REGION 1..97: note = O.33
SGAPRFLTCPKASVVSVGKDATLSSQIVGNPFPQVSWEKDKQPVTAGVRFRLAQDGDLYRLKILDCQLSDSGQYVSRARNAHGEAFACLGLQCDAEA

SEQ ID NO: 105 - protein, 9 aa, synthetic construct
  REGION 1..9: note = linker1
GGGGSGGGG

SEQ ID NO: 106 - protein, 5 aa, synthetic construct
  REGION 1..5: note = linker2
GGGGS

SEQ ID NO: 107 - protein, 227 aa, synthetic construct
  REGION 1..227: note = IgG1Fc(knob)
DKTHTCPPCPAPELLGGPSVFLFPPKPKDTLMISRTPEVTCVVVDVSHEDPEVKFNWYVDGVEVHNAKTKPREEQYNSTYRVVSVLTVLHQDWLNGKEYKCKVSNKALPAPIEKTISKAKGQPREPQVYTLPPCREEMTKNQVSLWCLVKGFYPSDIAVEWESNGQPENNYKTTPPVLDSDGSFFLYSKLTVDKSRWQQGNVFSCSVMHEALHNHYTQKSLSLSPGK

SEQ ID NO: 108 - protein, 227 aa, synthetic construct
  REGION 1..227: note = IgG1Fc(hole)
DKTHTCPPCPAPELLGGPSVFLFPPKPKDTLMISRTPEVTCVVVDVSHEDPEVKFNWYVDGVEVHNAKTKPREEQYNSTYRVVSVLTVLHQDWLNGKEYKCKVSNKALPAPIEKTISKAKGQPREPQVCTLPPSREEMTKNQVSLSCAVKGFYPSDIAVEWESNGQPENNYKTTPPVLDSDGSFFLVSKLTVDKSRWQQGNVFSCSVMHEALHNHYTQKSLSLSPGK

SEQ ID NO: 109 - protein, 5 aa, synthetic construct
  REGION 1..5: note = linker
ASTKG

SEQ ID NO: 110 - protein, 5 aa, synthetic construct
  REGION 1..5: note = linker
RTVAS

SEQ ID NO: 111 - protein, 227 aa, synthetic construct
  REGION 1..227: note = Fc1
DKTHTCPPCPAPEAAGGPSVFLFPPKPKDTLMISRTPEVTCVVVDVSHEDPEVKFNWYVDGVEVHNAKTKPREEQYNSTYRVVSVLTVLHQDWLNGKEYKCKVSNKALPAPIEKTISKAKGQPREPQVYTLPPCREEMTKNQVSLWCLVKGFYPSDIAVEWESNGQPENNYKTTPPVLDSDGSFFLYSKLTVDKSRWQQGNVFSCSVMHEALHNHYTQKSLSLSPGK

SEQ ID NO: 112 - protein, 227 aa, synthetic construct
  REGION 1..227: note = Fc2
DKTHTCPPCPAPEAAGGPSVFLFPPKPKDTLMISRTPEVTCVVVDVSHEDPEVKFNWYVDGVEVHNAKTKPREEQYNSTYRVVSVLTVLHQDWLNGKEYKCKVSNKALPAPIEKTISKAKGQPREPQVCTLPPSREEMTKNQVSLSCAVKGFYPSDIAVEWESNGQPENNYKTTPPVLDSDGSFFLVSKLTVDKSRWQQGNVFSCSVMHEALHNHYTQKSLSLSPGK

SEQ ID NO: 113 - protein, 103 aa, synthetic construct
  REGION 1..103: note = CH1
ASTKGPSVFPLAPSSKSTSGGTAALGCLVKDYFPEPVTVSWNSGALTSGVHTFPAVLQSSGLYSLSSVVTVPSSSLGTQTYICNVNHKPSNTKVDKKVEPKSC

SEQ ID NO: 114 - protein, 118 aa, synthetic construct
  REGION 1..118: note = VH2-L
QVQLVESGGGVVQPGRSLRLSCAASGFTFSSYTMHWVRQAPGKGLEWVTFISYDGNNKYYADSVKGRFTISRDNSKNTLYLQMNSLRAEDTAIYYCARTGWLGPFDYWGQGTLVTVSS

SEQ ID NO: 115 - protein, 108 aa, synthetic construct
  REGION 1..108: note = VL2-L
EIVLTQSPGTLSLSPGERATLSCRASQSVGSSYLAWYQQKPGQAPRLLIYGAFSRATGIPDRFSGSGSGTDFTLTISRLEPEDFAVYYCQQYGSSPWTFGQGTKVEIK

SEQ ID NO: 116-117 - skipped (2 entries)

SEQ ID NO: 118 - protein, 5 aa, synthetic construct
KAGIR

SEQ ID NO: 119 - protein, 5 aa, synthetic construct
DQPQF

SEQ ID NO: 120 - protein, 107 aa, Homo sapiens [sequence omitted]